European Patent Specification EP 3 006 570 B9, published October 4, 2023. Title: Method for determining the risk of developing an infectious disease. Applicant: Fundación para la Investigación Biomédica del Hospital Universitario La Paz Llamas Matías, Miguel Ángel. The sequence listing filed with the application follows.

SEQUENCE LISTING (4 sequences)

SEQ ID NO: 1 - DNA, 2313 bp, Homo sapiens
cacaagcgccgcgccatggacgcagccatcttggaccgggaacaaggcggcacttcgtcccgcccactccgcgtttagaccaattgcaaggcagcgaacctgaccgtgacgagccaatcagatcctgaggaaagttgaccgcgatagagtccttcgtcgcccaatcgtcgtctgtgtcccgcctcttcagtgacgcgaggcagaaccagccaatccctgcacggatagcgcccggaagaggctagaagctggattcagcgtgtccgcgacctcacctttaggtcctgtgaggtcggtggaatcctggggtcctccaaatctaccaggccatctccccagtttcccagttcttcctgcgtgcgggcgagagtggttgggccctcgggaacccactcagagcgaggctaaatttacggagggactttctgttagcagcatgagggcctgtggttagacctatagaggtatttcctttgatttaagccagaaagtcctgagagcggatcggggagcatttgcggatcggtcactttttcctcctttctgagtctcttatcccctaccacagggacggcccaggtggcaggatgtcctggtctggccttctccatggcctcaacacgtccctaacttgtggtaagtgggggacttgggcttcagggacgaggctagagggggagggttattcgctcttggacttgtgtgcctccgtcggagccccgagggaaacgggggtggaaaaacacggtggggttttggcagagctagggctgctagagcaagaggtgggaagcagctgcatggagggctactgcgtgtcaagcggcgtttgggtcagttttattatttatttatttaagatctccctctgtcgcccaggctgaagtgcagcggtgtgatcacagctcactgcagtctcgacctcctgggctcaagtgatcctcccgcctcagcctcccaagtagctgggaccacaggcctgcagaaccacaaccagctaactttttgattctttgtagagagggaggtctccctgtgtcgcccagtctggccttaactcctgagctcaagtgaccctccacagcctccaaaagtgctaggattacatgcatgagccactgagcctactattattttaaacagcattaaaaataatgcttcctggccagccgtggtggctcacgcctgtaatcccagcactttgagaggccgaggtcaggagttcgagaccagcctgaccaacatggtgaaaccccgtctctacttaaaaatacgaagattagccgagcgtggtggtgggtgcctgtagtcccagctgctcaggaggctgagacaggagaattgcttgaacccaggaggcagaggttgcagtgggccaagattgaggtactgcactccagcctgggcgacagagtgagactttgtctcaaaaaaaaaaaagaaaaaaaaaaaaaaggtaatgcttccttgaagaataaagagttacttttgtctgtagataacattagatgtgaacaaatgcatctttgtaaagtgctttaaacaatgcctaaaacaccaaaattgagttgctactactctaagatctgttctctgggataataacccctttcggccctctccaggcccagctctggttccccggctctgggctacctgctccatggctaccctgaaccagatgcaccgcctggggccccccaagcggccgcctcggaagctgggccccacggaaggccggccgcagctgaagggtgtggtcctgtgcacgtttacccgcaagccgaagaagcccaactcagccaatcgcaagtgctgtcgagtgcggctcagcactggccgcgaggccgtctgcttcatccctggggagggccacaccctgcaggagcaccagattgtccttgtggagggcggccgcacccaggacctgccaggcgtcaagctcaccgttgtgcgtggcaagtacgactgtggccacgtgcagaagaagtgacggctgggggcacagtgggctgggcgcccctgcagaacatgaaccttccgctcctggctgccacagggtcctccgatgctggcctttgcgcctctagaggcagccactcatggattcaagtcctggctccgcctcttccatcaggaccactattaagccataggagtcctgggggtgcaaagggtgcccctctgtcaacacccttggctcctgtgtttagaggggtggcctgaaggaccttttctgctgggacaagacactgtactgccctctgctgggaaggggttttaataaacagaccctggcgcttgtgatgtaaa

SEQ ID NO: 2 - DNA, 21 bp, Artificial sequence
  Sense primer for the detection of 12S rRNA
ccacgggaaacagcagtgatt

SEQ ID NO: 3 - DNA, 25 bp, Artificial sequence
  Antisense primer for the detection of 12S rRNA
ctattgacttgggttaatcgtgtga

SEQ ID NO: 4 - DNA, 14 bp, Artificial sequence
  Probe for the detection of 12S rRNA
tgccagccaccgcg